European Patent Specification EP 3 231 864 B1, published July 31, 2024. Title: MODIFIED IMMUNE CELL, METHOD FOR PRODUCING THE MODIFIED IMMUNE CELL, AND USE THEREOF. Applicant: RIKEN. The sequence listing filed with the application follows.

SEQUENCE LISTING (2 sequences)

SEQ ID NO: 1 - DNA, 831 bp, Homo sapiens
atgaaaaagcatctgacgaccttcttggtgattttgtggctttatttttatagggggaatggcaaaaaccaagtggagcagagtcctcagtccctgatcatcctggagggaaagaactgcactcttcaatgcaattatacagtgagccccttcagcaacttaaggtggtataagcaagatactgggagaggtcctgtttccctgacaatcatgactttcagtgagaacacaaagtcgaacggaagatatacagcaactctggatgcagacacaaagcaaagctctctgcacatcacagcctcccagctcagcgattcagcctcctacatctgtgtggtgagcgacagaggctcaaccctggggaggctatactttggaagaggaactcagttgactgtctggcctgatatccagaaccctgaccctgccgtgtaccagctgagagactctaaatccagtgacaagtctgtctgcctattcaccgattttgattctcaaacaaatgtgtcacaaagtaaggattctgatgtgtatatcacagacaaaactgtgctagacatgaggtctatggacttcaagagcaacagtgctgtggcctggagcaacaaatctgactttgcatgtgcaaacgccttcaacaacagcattattccagaagacaccttcttccccagcccagaaagttcctgtgatgtcaagctggtcgagaaaagctttgaaacagatacgaacctaaactttcaaaacctgtcagtgattgggttccgaatcctcctcctgaaagtggccgggtttaatctgctcatgacgctgcggctgtggtccagctga

SEQ ID NO: 2 - DNA, 933 bp, Homo sapiens
atgactatcaggctcctctgctacatgggcttttattttctgggggcaggcctcatggaagctgacatctaccagaccccaagataccttgttatagggacaggaaagaagatcactctggaatgttctcaaaccatgggccatgacaaaatgtactggtatcaacaagatccaggaatggaactacacctcatccactattcctatggagttaattccacagagaagggagatctttcctctgagtcaacagtctccagaataaggacggagcattttcccctgaccctggagtctgccaggccctcacatacctctcagtacctctgtgccagcgagcagagggggggagtagatgaaaaactgttttttggcagtggaacccagctctctgtcttggaggacctgaacaaggtgttcccacccgaggtcgctgtgtttgagccatcagaagcagagatctcccacacccaaaaggccacactggtgtgcctggccacaggcttcttccctgaccacgtggagctgagctggtgggtgaatgggaaggaggtgcacagtggggtcagcacggacccgcagcccctcaaggagcagcccgccctcaatgactccagatactgcctgagcagccgcctgagggtctcggccaccttctggcagaacccccgcaaccacttccgctgtcaagtccagttctacgggctctcggagaatgacgagtggacccaggatagggccaaacccgtcacccagatcgtcagcgccgaggcctggggtagagcagactgtggctttacctcggtgtcctaccagcaaggggtcctgtctgccaccatcctctatgagatcctgctagggaaggccaccctgtatgctgtgctggtcagcgcccttgtgttgatggccatggtcaagagaaaggatttctga